European Patent Specification EP 3 784 267 B1, published November 12, 2025. Title: Integrin Targeting Ligands and Uses Thereof. Applicant: ARROWHEAD PHARMACEUTICALS, INC. The sequence listing filed with the application follows.

SEQUENCE LISTING (9 sequences)

SEQ ID NO: 1 - RNA, 21 nt, Homo sapiens
  RNAi agent antisense strand modified sequence
uuucaugaaaucguuacguug

SEQ ID NO: 2 - RNA, 21 nt, Artificial sequence
  RNAi agent sense strand modified sequence
caacguaacgauuucaugaaa

SEQ ID NO: 3 - RNA, 21 nt, Artificial sequence
  RNAi agent sense strand modified sequence
caacguaacgauuucaugaaa

SEQ ID NO: 4 - RNA, 21 nt, Artificial sequence
  RNAi agent sense strand modified sequence
caacguaacgauuucaugaaa

SEQ ID NO: 5 - RNA, 21 nt, Artificial sequence
  RNAi agent sense strand modified sequence
caacguaacgauuucaugaaa

SEQ ID NO: 6 - RNA, 21 nt, Artificial sequence
  RNAi agent sense strand modified sequence
caacguaacgauuucaugaaa

SEQ ID NO: 7 - RNA, 21 nt, Artificial sequence
  RNAi agent sense strand modified sequence
caacguaacgauuucaugaaa

SEQ ID NO: 8 - RNA, 21 nt, Artificial sequence
  RNAi agent sense strand modified sequence
caacguaacgauuucaugaaa

SEQ ID NO: 9 - RNA, 21 nt, Artificial sequence
  RNAi agent sense strand modified sequence
caacguaacgauuucaugaaa